European Patent Application EP 4 549 462 A1, published May 7, 2025. Title: Procollagen I N-Terminal Propeptide-specific antibody, kit and use thereof. Applicant: Shenzhen Mindray Bio-Medical Electronics Co., Ltd. Application EP. The sequence listing filed with the application follows.

SEQUENCE LISTING (85 sequences)

SEQ ID NO: 1 - protein, 5 aa, synthetic construct
  source 1..5: note = PINP01 Kabat CDR-H1 amino acid sequence
SYWMN

SEQ ID NO: 2 - protein, 17 aa, synthetic construct
  source 1..17: note = PINP01 Kabat CDR-H2 amino acid sequence
MIHPSDSETRLNQKFKD

SEQ ID NO: 3 - protein, 9 aa, synthetic construct
  source 1..9: note = PINP01 Kabat CDR-H3 amino acid sequence
THIYYVFDY

SEQ ID NO: 4 - protein, 17 aa, synthetic construct
  source 1..17: note = PINP01 Kabat CDR-L1 amino acid sequence
KSSQSLLNSRTRKNYLA

SEQ ID NO: 5 - protein, 7 aa, synthetic construct
  source 1..7: note = PINP01 Kabat CDR-L2 amino acid sequence
WASTRES

SEQ ID NO: 6 - protein, 8 aa, synthetic construct
  source 1..8: note = PINP01 Kabat CDR-L3 amino acid sequence
KQSYNLYT

SEQ ID NO: 7 - protein, 5 aa, synthetic construct
  source 1..5: note = hPINP02 Kabat CDR-H1 amino acid sequence
NAAMY

SEQ ID NO: 8 - protein, 19 aa, synthetic construct
  source 1..19: note = hPINP02 Kabat CDR-H2 amino acid sequence
RIRTKPNNYATYYADSVKG

SEQ ID NO: 9 - protein, 10 aa, synthetic construct
  source 1..10: note = hPINP02 Kabat CDR-H3 amino acid sequence
TTTDMGPMGY

SEQ ID NO: 10 - protein, 11 aa, synthetic construct
  source 1..11: note = hPINP02 Kabat CDR-L1 amino acid sequence
RASQDIGNYLR

SEQ ID NO: 11 - protein, 7 aa, synthetic construct
  source 1..7: note = hPINP02 Kabat CDR-L2 amino acid sequence
GETNLAN

SEQ ID NO: 12 - protein, 9 aa, synthetic construct
  source 1..9: note = hPINP02 Kabat CDR-L3amino acid sequence
LQHYDYPLT

SEQ ID NO: 13 - protein, 5 aa, synthetic construct
  source 1..5: note = hPINP03 Kabat CDR-H1 amino acid sequence
NNGVS

SEQ ID NO: 14 - protein, 16 aa, synthetic construct
  source 1..16: note = hPINP03 Kabat CDR-H2 amino acid sequence
AMSSGGNTYYNSGLKS

SEQ ID NO: 15 - protein, 7 aa, synthetic construct
  source 1..7: note = hPINP03 Kabat CDR-H3 amino acid sequence
HDAGLIY

SEQ ID NO: 16 - protein, 11 aa, synthetic construct
  source 1..11: note = hPINP03 Kabat CDR-L1 amino acid sequence
KASQNVGTNVD

SEQ ID NO: 17 - protein, 7 aa, synthetic construct
  source 1..7: note = hPINP03 Kabat CDR-L2 amino acid sequence
GASNRYT

SEQ ID NO: 18 - protein, 9 aa, synthetic construct
  source 1..9: note = hPINP03 Kabat CDR-L3 amino acid sequence
LQYNDTPWT

SEQ ID NO: 19 - protein, 5 aa, synthetic construct
  source 1..5: note = hPINP04 Kabat CDR-H1 amino acid sequence
DYYMA

SEQ ID NO: 20 - protein, 17 aa, synthetic construct
  source 1..17: note = hPINP04 Kabat CDR-H2 amino acid sequence
TISYDGSGTHYRDSVKG

SEQ ID NO: 21 - protein, 12 aa, synthetic construct
  source 1..12: note = hPINP04 Kabat CDR-H3 amino acid sequence
RRGYGYYYVMDA

SEQ ID NO: 22 - protein, 11 aa, synthetic construct
  source 1..11: note = hPINP04 Kabat CDR-L1 amino acid sequence
KASQNVGSNVD

SEQ ID NO: 23 - protein, 7 aa, synthetic construct
  source 1..7: note = hPINP04 Kabat CDR-L2 amino acid sequence
KASNLYT

SEQ ID NO: 24 - protein, 9 aa, synthetic construct
  source 1..9: note = hPINP04 Kabat CDR-L3 amino acid sequence
MQSGSYPPT

SEQ ID NO: 25 - protein, 5 aa, synthetic construct
  source 1..5: note = hPINP05 Kabat CDR-H1 amino acid sequence
NAAMY

SEQ ID NO: 26 - protein, 19 aa, synthetic construct
  source 1..19: note = hPINP05 Kabat CDR-H2 amino acid sequence
RIRTKVNNYATYYADSVRG

SEQ ID NO: 27 - protein, 17 aa, synthetic construct
  source 1..17: note = hPINP05 Kabat CDR-H3 amino acid sequence
AGYYDGTYYYEGDYFDY

SEQ ID NO: 28 - protein, 15 aa, synthetic construct
  source 1..15: note = hPINP05 Kabat CDR-L1 amino acid sequence
RASQSVSITGYSLMH

SEQ ID NO: 29 - protein, 7 aa, synthetic construct
  source 1..7: note = hPINP05 Kabat CDR-L2 amino acid sequence
RTSDLAS

SEQ ID NO: 30 - protein, 9 aa, synthetic construct
  source 1..9: note = hPINP05 Kabat CDR-L3 amino acid sequence
QQSRESPPT

SEQ ID NO: 31 - protein, 5 aa, synthetic construct
  source 1..5: note = hPINP06 Kabat CDR-H1 amino acid sequence
NAAMY

SEQ ID NO: 32 - protein, 19 aa, synthetic construct
  source 1..19: note = hPINP06 Kabat CDR-H2 amino acid sequence
RIRTKPNDYATYYTDSVKG

SEQ ID NO: 33 - protein, 10 aa, synthetic construct
  source 1..10: note = hPINP06 Kabat CDR-H3 amino acid sequence
ETRNLDWFAY

SEQ ID NO: 34 - protein, 16 aa, synthetic construct
  source 1..16: note = hPINP06 Kabat CDR-L1 amino acid sequence
RSSKSPRHSNGITYVY

SEQ ID NO: 35 - protein, 7 aa, synthetic construct
  source 1..7: note = hPINP06 Kabat CDR-L2 amino acid sequence
RMSNLAS

SEQ ID NO: 36 - protein, 9 aa, synthetic construct
  source 1..9: note = hPINP06 Kabat CDR-L3 amino acid sequence
GQVLENLPT

SEQ ID NO: 37 - protein, 7 aa, synthetic construct
  source 1..7: note = hPINP07 Kabat CDR-H1 amino acid sequence
GSSVGVG

SEQ ID NO: 38 - protein, 16 aa, synthetic construct
  source 1..16: note = hPINP07 Kabat CDR-H2 amino acid sequence
TIGWEDVKHYNPSLKS

SEQ ID NO: 39 - protein, 7 aa, synthetic construct
  source 1..7: note = hPINP07 Kabat CDR-H3 amino acid sequence
SWERFDY

SEQ ID NO: 40 - protein, 11 aa, synthetic construct
  source 1..11: note = hPINP07 Kabat CDR-L1 amino acid sequence
SGDELPKRYAY

SEQ ID NO: 41 - protein, 7 aa, synthetic construct
  source 1..7: note = hPINP07 Kabat CDR-L2 amino acid sequence
KDSERPS

SEQ ID NO: 42 - protein, 11 aa, synthetic construct
  source 1..11: note = hPINP07 Kabat CDR-L3 amino acid sequence
HSTYSDDKLPV

SEQ ID NO: 43 - protein, 179 aa, synthetic construct
  source 1..179: note = A1-PINP
MFSFVDLRLLLLLAATALLTHGQEEGQVEGQDEDIPPITCVQNGLRYHDRDVWKPEPCRICVCDNGKVLCDDVICDETKNCPGAEVPEGECCPVCPDGSESPTDQETTGVEGPKGDTGPRGPRGPAGPPGRDGIPGQPGLPGPPGPPGPPGPPGLGGNFAPGGGSGGGSGGGSHHHHHH

SEQ ID NO: 44 - DNA, 15 bp, synthetic construct
  source 1..15: mol_type = other DNA; note = PINP01 Kabat CDR-H1 nucleotide sequence
agctactggatgaac

SEQ ID NO: 45 - DNA, 51 bp, synthetic construct
  source 1..51: mol_type = other DNA; note = PINP01 Kabat CDR-H2 nucleotide sequence
atgattcatccttccgatagtgaaactaggttaaatcagaagttcaaggac

SEQ ID NO: 46 - DNA, 27 bp, synthetic construct
  source 1..27: mol_type = other DNA; note = PINP01 Kabat CDR-H3 nucleotide sequence
acccacatctactatgtctttgactac

SEQ ID NO: 47 - DNA, 51 bp, synthetic construct
  source 1..51: mol_type = other DNA; note = PINP01 Kabat CDR-L1 nucleotide sequence
aaatccagtcagagtctgctcaacagtagaacccgaaagaactacttggct

SEQ ID NO: 48 - DNA, 21 bp, synthetic construct
  source 1..21: mol_type = other DNA; note = PINP01 Kabat CDR-L2 nucleotide sequence
tgggcatccactagggaatct

SEQ ID NO: 49 - DNA, 24 bp, synthetic construct
  source 1..24: mol_type = other DNA; note = PINP01 Kabat CDR-L3 nucleotide sequence
aagcaatcttataatctgtacacg

SEQ ID NO: 50 - DNA, 15 bp, synthetic construct
  source 1..15: mol_type = other DNA; note = hPINP02 Kabat CDR-H1 nucleotide sequence
aatgctgccatgtac

SEQ ID NO: 51 - DNA, 57 bp, synthetic construct
  source 1..57: mol_type = other DNA; note = hPINP02 Kabat CDR-H2 nucleotide sequence
cgcataagaactaaacctaataattatgcaacatattatgctgattcagtgaaaggc

SEQ ID NO: 52 - DNA, 30 bp, synthetic construct
  source 1..30: mol_type = other DNA; note = hPINP02 Kabat CDR-H3 nucleotide sequence
acgactacggatatgggtcctatggggtac

SEQ ID NO: 53 - DNA, 33 bp, synthetic construct
  source 1..33: mol_type = other DNA; note = hPINP02 Kabat CDR-L1 nucleotide sequence
cgggcaagtcaagacattggaaattatttaaga

SEQ ID NO: 54 - DNA, 21 bp, synthetic construct
  source 1..21: mol_type = other DNA; note = hPINP02 Kabat CDR-L2 nucleotide sequence
ggtgaaaccaacttggcaaat

SEQ ID NO: 55 - DNA, 27 bp, synthetic construct
  source 1..27: mol_type = other DNA; note = hPINP02 Kabat CDR-L3 nucleotide sequence
ctgcagcattatgattatcctctcacg

SEQ ID NO: 56 - DNA, 15 bp, synthetic construct
  source 1..15: mol_type = other DNA; note = hPINP03 Kabat CDR-H1 nucleotide sequence
aacaatggtgtaagc

SEQ ID NO: 57 - DNA, 48 bp, synthetic construct
  source 1..48: mol_type = other DNA; note = hPINP03 Kabat CDR-H2 nucleotide sequence
gcaatgtcaagtggtggaaacacatattataattcaggtctcaaatcc

SEQ ID NO: 58 - DNA, 21 bp, synthetic construct
  source 1..21: mol_type = other DNA; note = hPINP03 Kabat CDR-H3 nucleotide sequence
cacgacgcggggctaatttac

SEQ ID NO: 59 - DNA, 33 bp, synthetic construct
  source 1..33: mol_type = other DNA; note = hPINP03 Kabat CDR-L1 nucleotide sequence
aaggccagtcagaatgtgggtactaatgtagac

SEQ ID NO: 60 - DNA, 21 bp, synthetic construct
  source 1..21: mol_type = other DNA; note = hPINP03 Kabat CDR-L2 nucleotide sequence
ggggcatccaaccggtacact

SEQ ID NO: 61 - DNA, 27 bp, synthetic construct
  source 1..27: mol_type = other DNA; note = hPINP03 Kabat CDR-L3 nucleotide sequence
ctacagtataacgacactccgtggacg

SEQ ID NO: 62 - DNA, 15 bp, synthetic construct
  source 1..15: mol_type = other DNA; note = hPINP04 Kabat CDR-H1 nucleotide sequence
gactattacatggcc

SEQ ID NO: 63 - DNA, 51 bp, synthetic construct
  source 1..51: mol_type = other DNA; note = hPINP04 Kabat CDR-H2 nucleotide sequence
accattagttatgatggtagtggcactcactatcgagactccgtgaagggc

SEQ ID NO: 64 - DNA, 36 bp, synthetic construct
  source 1..36: mol_type = other DNA; note = hPINP04 Kabat CDR-H3 nucleotide sequence
cgaaggggttacggctattactatgttatggatgcc

SEQ ID NO: 65 - DNA, 33 bp, synthetic construct
  source 1..33: mol_type = other DNA; note = hPINP04 Kabat CDR-L1 nucleotide sequence
aaggccagtcaaaatgtgggttctaatgtagac

SEQ ID NO: 66 - DNA, 21 bp, synthetic construct
  source 1..21: mol_type = other DNA; note = hPINP04 Kabat CDR-L2 nucleotide sequence
aaagcatccaacctgtacacg

SEQ ID NO: 67 - DNA, 27 bp, synthetic construct
  source 1..27: mol_type = other DNA; note = hPINP04 Kabat CDR-L3 nucleotide sequence
atgcagtctggctcctatcctccaacg

SEQ ID NO: 68 - DNA, 15 bp, synthetic construct
  source 1..15: mol_type = other DNA; note = hPINP05 Kabat CDR-H1 nucleotide sequence
aatgctgccatgtac

SEQ ID NO: 69 - DNA, 57 bp, synthetic construct
  source 1..57: mol_type = other DNA; note = hPINP05 Kabat CDR-H2 nucleotide sequence
cgcataagaactaaagttaataattatgcaacatattatgctgattcagtgagaggc

SEQ ID NO: 70 - DNA, 51 bp, synthetic construct
  source 1..51: mol_type = other DNA; note = hPINP05 Kabat CDR-H3 nucleotide sequence
gcgggctattatgatggtacttattattacgagggcgactactttgattac

SEQ ID NO: 71 - DNA, 45 bp, synthetic construct
  source 1..45: mol_type = other DNA; note = hPINP05 Kabat CDR-L1 nucleotide sequence
agggccagccaaagtgtcagtataactggatatagtcttatgcac

SEQ ID NO: 72 - DNA, 21 bp, synthetic construct
  source 1..21: mol_type = other DNA; note = hPINP05 Kabat CDR-L2 nucleotide sequence
cgtacatccgacctagcatct

SEQ ID NO: 73 - DNA, 27 bp, synthetic construct
  source 1..27: mol_type = other DNA; note = hPINP05 Kabat CDR-L3 nucleotide sequence
cagcagagtagggagtctcctccgacg

SEQ ID NO: 74 - DNA, 15 bp, synthetic construct
  source 1..15: mol_type = other DNA; note = hPINP06 Kabat CDR-H1 nucleotide sequence
aatgctgccatgtac

SEQ ID NO: 75 - DNA, 57 bp, synthetic construct
  source 1..57: mol_type = other DNA; note = hPINP06 Kabat CDR-H2 nucleotide sequence
cgcataagaactaaacctaatgattatgcaacatattacactgattcagtgaaaggc

SEQ ID NO: 76 - DNA, 30 bp, synthetic construct
  source 1..30: mol_type = other DNA; note = hPINP06 Kabat CDR-H3 nucleotide sequence
gagactcgcaacttggattggtttgcttac

SEQ ID NO: 77 - DNA, 48 bp, synthetic construct
  source 1..48: mol_type = other DNA; note = hPINP06 Kabat CDR-L1 nucleotide sequence
agatctagtaagagtccgcgacatagtaatggcatcacttacgtgtat

SEQ ID NO: 78 - DNA, 21 bp, synthetic construct
  source 1..21: mol_type = other DNA; note = hPINP06 Kabat CDR-L2 nucleotide sequence
cggatgtccaaccttgcctca

SEQ ID NO: 79 - DNA, 27 bp, synthetic construct
  source 1..27: mol_type = other DNA; note = hPINP06 Kabat CDR-L3 nucleotide sequence
ggacaggttctagaaaatcttccgacg

SEQ ID NO: 80 - DNA, 21 bp, synthetic construct
  source 1..21: mol_type = other DNA; note = hPINP07 Kabat CDR-H1 nucleotide sequence
ggttccagtgtgggcgtgggc

SEQ ID NO: 81 - DNA, 48 bp, synthetic construct
  source 1..48: mol_type = other DNA; note = hPINP07 Kabat CDR-H2 nucleotide sequence
accattgggtgggaggatgttaagcactacaatccatctctgaagagc

SEQ ID NO: 82 - DNA, 21 bp, synthetic construct
  source 1..21: mol_type = other DNA; note = hPINP07 Kabat CDR-H3 nucleotide sequence
tcctgggagaggtttgattac

SEQ ID NO: 83 - DNA, 33 bp, synthetic construct
  source 1..33: mol_type = other DNA; note = hPINP07 Kabat CDR-L1 nucleotide sequence
tctggagatgagttaccaaaaagatatgcttat

SEQ ID NO: 84 - DNA, 21 bp, synthetic construct
  source 1..21: mol_type = other DNA; note = hPINP07 Kabat CDR-L2 nucleotide sequence
aaagatagtgagcggccctca

SEQ ID NO: 85 - DNA, 33 bp, synthetic construct
  source 1..33: mol_type = other DNA; note = hPINP07 Kabat CDR-L3 nucleotide sequence
cactcgacatatagtgatgataaactccctgtt